European Patent Application EP 4 141 102 A1, published March 1, 2023. Title: A nucleic acid capable of interacting with Endocrine disruptor receptor and a use the same. Applicant: KUMIAI CHEMICAL INDUSTRY CO., LTD. University Public Corporation Osaka. The sequence listing filed with the application follows.

SEQUENCE LISTING (54 sequences)

SEQ ID NO: 1 - DNA, 16 bp, Artificial
  Synthetic DNA
  misc_feature (7)..(10): n is a, c, g, or t
cacgcgnnnncacgtg

SEQ ID NO: 2 - DNA, 43 bp, Daphnia magna
caaagaaaatacgcacacgcggcggcacgtgtgtgcatcccat

SEQ ID NO: 3 - DNA, 49 bp, Artificial
  Synthetic DNA
ctagtcaaagaaaatacgcacacgcggcggcacgtgtgtgcatcccatt

SEQ ID NO: 4 - DNA, 49 bp, Artificial
  Synthetic DNA
ctagaatgggatgcacacacgtgccgccgcgtgtgcgtattttctttga

SEQ ID NO: 5 - DNA, 54 bp, Daphnia magna
caaagaaaatacgcacacgcggcggcacgtgtgtgcatcccatcttccgttcgg

SEQ ID NO: 6 - DNA, 60 bp, Artificial
  Synthetic DNA
ctagtcaaagaaaatacgcacacgcggcggcacgtgtgtgcatcccatcttccgttcggt

SEQ ID NO: 7 - DNA, 60 bp, Artificial
  Synthetic DNA
ctagaccgaacggaagatgggatgcacacacgtgccgccgcgtgtgcgtattttctttga

SEQ ID NO: 8 - DNA, 30 bp, Daphnia magna
atacgcacacgcggcggcacgtgtgtgcat

SEQ ID NO: 9 - DNA, 36 bp, Artificial
  Synthetic DNA
ctagtatacgcacacgcggcggcacgtgtgtgcatt

SEQ ID NO: 10 - DNA, 36 bp, Artificial
  Synthetic DNA
ctagaatgcacacacgtgccgccgcgtgtgcgtata

SEQ ID NO: 11 - DNA, 2088 bp, Daphnia magna
  CDS (1)..(2088)
atggacaaaatgagcgagacattaccaagttcgagccgggagatgcggaatcgtgcggagaagcaacggcgtgacaagctcaatgcctacatttcggagctttatagtctcgttccgtcagcggctgccgcccctaggaagctggacaagacgagcacgctccgtctttcggcaaattttttgcgcatccatcaaaatatggatctacgaatgaagccgtacaaccgatggaatgctttagctggtcattcaatcttagagaaattggactcctttttgcttgtcgtctcgtgctgctctggcaagatcatctacgtcacggatcgagtggagaaattgctcggacatgcgcaggtcgatatgatgggctaccagttatcctgttttgtccaccaggcagatcaagatgcaattgaaaaacggctcagtgcttttgctgcacaagtggctgctaatccagatgcttcagattctgccgatggacaagtctattcattcgaatgtcgcctagccggacgccaactcagtcggggcgaaccgaccgtctatgaacgggtcagtgtctcagggacttttcgaggccctcggagaagacgtgactgggctgatctcaaaagcagtgatagatctgtggcaactgttcaacaacacaacgactacagcgagccgctttttattggcttggtgcgcattttacaaacacccaacactttacctccattgacgatcatgcaagctgttcaggacgagtatatcactcagcacacaaccggtggcaccattatacaaaccgatcatcgcatcgccatcattgctggttatctgagtggcgaggtgacgggcatgtcagcatacgattatgtttatagcgaagatttggagtacactctcaaagctcaaagcctcatgttaactcggagtgaaggaatggtgacttatcgcctaaaaaccagtacgggtcgtttgattttccttcgatcaagaggtttcatccaatacgatgaaaacacgaaggaaattgtcagcttcttctgcatcaattcactcatcgacgaagagcaaggaatgaaggaaatgcaggaaatgcgggccatgttagacaaacttaacattgcaactgttacgccagcgatagcgtcatcgccaacgagcacgattgaaccagttggagcagcttctactcaagagccactttctcgttgtgttcgggcgtcagtggggaaaccaccgccttctttttcttctaatggctgccaccttgcgaatgggtctagggtctcgggcctgcctagatccagtattatgcccaacggacataacagtttatgcatttcaccctcctctgaacttcagtactccccttcaggatcgtcttcgtcttctttcagtgaagaacgttgccaatcttctacaccgcattcgctcgtgtcatctcccatggaaattcctaatttagttgctgtttcctacccatttgcacccatacctttcccatggcgaccatcgacagactgttctccgatcaccacgacatctaacggtcacgttaacactagagaagttagcaaatcccccgatgtcgatcagagcgatcctcttggtgaaccaggattgctggctcttacgctggatcatcaatgggaaacggctcccaatagtcagagcatgatcgtccagcacaatgggccacaaagtcatcagcagtccttggtagccgtcagtccccttcaagctcatttgcttcagtcatcgccaaacgataacatagaaccgattcggtccaccctgaaatcgccgccatcgtccaccagctgtcccgttcaacctccccaccaatatcaggaagatgctctgaaaatctcgattcccgatcgttgtccgacgaatgaactgagtcgaaacaactgtctcaacggctacatcatttggcctcaaaagatgtcgcccaaaaatcgaaaggagaatcttatattgtcgtacttggacgtcgacaagcatgcctacaaacagccagagattaccggaactgctgaccagcactactatcatagtgatttaaaagtgaatgctggaaccaacagtgcatag

SEQ ID NO: 12 - protein, 695 aa, Daphnia magna
MDKMSETLPSSSREMRNRAEKQRRDKLNAYISELYSLVPSAAAAPRKLDKTSTLRLSANFLRIHQNMDLRMKPYNRWNALAGHSILEKLDSFLLVVSCCSGKIIYVTDRVEKLLGHAQVDMMGYQLSCFVHQADQDAIEKRLSAFAAQVAANPDASDSADGQVYSFECRLAGRQLSRGEPTVYERVSVSGTFRGPRRRRDWADLKSSDRSVATVQQHNDYSEPLFIGLVRILQTPNTLPPLTIMQAVQDEYITQHTTGGTIIQTDHRIAIIAGYLSGEVTGMSAYDYVYSEDLEYTLKAQSLMLTRSEGMVTYRLKTSTGRLIFLRSRGFIQYDENTKEIVSFFCINSLIDEEQGMKEMQEMRAMLDKLNIATVTPAIASSPTSTIEPVGAASTQEPLSRCVRASVGKPPPSFSSNGCHLANGSRVSGLPRSSIMPNGHNSLCISPSSELQYSPSGSSSSSFSEERCQSSTPHSLVSSPMEIPNLVAVSYPFAPIPFPWRPSTDCSPITTTSNGHVNTREVSKSPDVDQSDPLGEPGLLALTLDHQWETAPNSQSMIVQHNGPQSHQQSLVAVSPLQAHLLQSSPNDNIEPIRSTLKSPPSSTSCPVQPPHQYQEDALKISIPDRCPTNELSRNNCLNGYIIWPQKMSPKNRKENLILSYLDVDKHAYKQPEITGTADQHYYHSDLKVNAGTNSA

SEQ ID NO: 13 - DNA, 6672 bp, Daphnia magna
  CDS (1)..(6672)
atgctgacggataccgcattcctggatgatgcacagagtttgggtgcaattccatgcgagtcactatcgtccgagccgtgctgggccaacatgaatacgctcagcagcggcggcggaggtggtggcggcagcggtggtagcagcaatagcaacagcccaggtctcggcagcaacaacaacaatcatacgacgtcgtcggcctcaccgacgacgacgacgacgaccggcaacagcaacagcagcggcggtggcgctggcggcagcaacggcctcaccggcacctcggcggccgccatcaaaaagcgacgcaaatccgacacgaagccgctgtcgcaaatcaacaagtgtctcaacgaaaaaagacgtcgcgaacaggaaaacgtctacattgaagagttggctgaattgatttcggtgagcattgccgacgtgaactcgctgtctgtgaaaccggacaagtgcgccattttacaagagacggtcaatcagatccgaaagatccgtgaacaggaagaagacggacgaagttcgagtagcagtagtagcagcagcagcagcaccagttcgaatggtagtagcaccaacagttctggcacgagttcagccaatagcggaacaggaggaaccgtaggagctgtaggggcaggaggagcaggaggagccgtaggagccgtaggagccgtaggaggaggtggacagggcaacaacacgacgtcgcccggcggagtgactgatggcggcgtcgggccgctgctccaacagggcgacgtttcatcatcgaaaccggccctgctagacacgcaacttttgggtacgttcctgctcgaagcccttgacggcttcctgtttgtcgtcaacacggaagggaaaacggagtatgtctctgaaaatgtcgcccattttctacactaccaaccgcaagatctcgtcggcaaatccatctacaattttatccaccacggagatcacgcccgtttttcgtcgtcgctcttacccacggccatcgcgtggccgagtgaaatggcaccaacgtctcagaacaggataggtcgctgtttcaattgccgattactgatccagccgcttggcgagcaagacgaaacgatggaggagaagcagcagcgagtcgaacactatgagaacatgcaaatatctgccgttctccagccgtatccagcggacggtggccagcagcagcagcagccaacaaagaaaatcagcggggcagcggcagctgcggccgcagccgcagccgccgtcggcttggagacgtccgatttggaactggcgctgacgtctgtggctagcggctcgctcgcaggtgatccgcagcactgcctcgtgtgcgtagccaggcgcattccgtcgacggagaaaatggctgccgccaacccgacggttggaggtccaatcgtggaacagttcaccaccaaattggacccgagtggcaagatagtagccgtcgatgtgacgggcgtttcttcgccctacagttcctacttgagcaaagaggcgctcgtctcgtgtacgatccaggagctctgctaccccgacgatttgcccgttttccaggcgcatctacaggaaacgctgcattccggctgcggcatcagctccagatatcggctcagattgaccggcgcctccaccccgatgggtcaccgtggtggcgccggcggaggcagcggaggctttctcgtcgttcaaaccaagtcgaaacgtttcattcacggtgacacgcacgagacggactttatcatggccacgcattccatcatcgtcgatgacgacggtgaagatgtcgacactggcaacagcagcagcagcaacaccaacaccaacaccagccgaatgatgttgttggcggccgcgagcgacacgctcaacgaccatcaccgtctatcggaatcgacgggcagtatcatcagtcagccgcagcaacagcagcaacagcagcagcagcagcagcagcagcagcagagcaacccggtgctcaccagcgtcgtccgccacgatgtgatatcagccaccagtttcggcaacagcggctgcagtggtggcgccacgacggcaaccacttcctccacctcctcctcctcctactccagtaccttcgccggactcagtctgggaacgagcggcgatcttctcaatgactttgtcgtgcccgacttgttcatggcttcaccgccctgggatttcaataacagcgagtcgagcctggacgacggcggcagcggcgtcgcgctggccgccgcctcggctgccgcttcggccgctgttgccgccgctgctcaaatcaccaacagtcaccacttgcaggccgtcacggccacgtccagcctgcagctctcggttccgtcgcctctctccctcatcccgtcgggcggtcctctcttggccggccacctaccccatcattctgttggcggaatgatcaactggggcagccctccgccgtcggccggtgccgggggagtaggacaacgagccggctcgacaccgtgcggacaaatggcgaccgtcatgggctcgtcgaggcccagctcgagacaaagcgcctcgtcgacaccgcgaccgcccagcgtgtcttcagccttcagtccggctcccaattccgtcctgggcgtcgttcatccgtcacccgtgctcagtccagtcggcgccaccagcatccattcagccgcaatgtcttgcaccagcggtttggtcactggctccacgtcgtcgtcatcggctggccagcaacaacccagtccggccagtatgacgacaccctttagcaacaatttcccgttcagtccactccaagatcccattcctcagcatccggcaacggctccgcagacccataatccggccacccctttcctggacgaagtccgtgacaccaaggacggaatcatctcgtccggccctggtggtagtgttagccacggtcacaactacctgtctggtggatctcaccaccagcagcagcatcatcatcatcatcaacaacaacaacagcaacaacaacagcaacaacacgcgaccgacaaacaaatgagcgctctcagtagtttattgaactgtaacgacgctgccacatcatcgtcgtcgtcttcgtcgtcctcttcgtcttcttcatcttcttcctcgttggccgaatctggccggttacgcattttgctcatgcaaagaccgggcaacgctccgccaccctcagcccatcagcagccaggtcattctagcagtggtagtagtagtagtagtagtagtacaagtacaagtacaagtacaagtacaagtacaagtacaaatacaaatacaaatactaatagtagcaacaacaataacaacaacaacaacaacgctagcggcaacaacaacagcagtagtgtcaacgggagccatctgttggcggctttgggcgacgctgaggccgtcaaacgcgaaaaagatgaaaatagcggtgcgccctcttgtggctcgttgagcgtcaccaaaggcagtcacggcaaccgcattctcaaagggttgctgaaccaggacgatggcgatgaagctgatcaagcggacgatacgagcaatcatcgcttcttgttgacggccagaggcaacctttctggagacggagtcaagaccagtagtagcgcgggcaacaacaacaacaacaccaccaacaccaacaacaataacaccaacaacaacaacaacatgctgcacaaattgttgaatgtgcggagcgacgacgatgccgagcagcggatgggtctgcgcaagcccaacgaattgctcaagaaacttctcaaggaccccgaagaggatcaccaacaggcaagtggaaacggcagcagcagtgcctgtggcggcaccggaagcggtggcacggccaaccagctccaacaatttcaccaccaacgtcaacagcagcagcagcaacaacagcaacaccagcaacaccagcaacaccagcaacaccaacaaagtcagcagcaacagcaacagaatcaacatcatcattcagatcaggtgtcgttccaggaagagcaattactgaaatcgtttggtttcccatcaccgacagcctcgtcaggttcgtctacggcagcaacggttgcaacgggatctttggccaacatgttggctaccagtcaaatgactcatctcagatctcctcaaccgccaggcatgtcgagccattgcgacggattgttggagtttggcggagttgtttgtagcagtacgaccgccagtggcatggtgtttggtggcaatgctgccgttggtggagctagtgggatgcggggcacgaaaaggcacagcgaagaagctcgtgacgaggtgaaagccagcaaagagcccatgctgagcgccgaccacctgatgatgtccgcaggcggaggcggggtcttgcaccagctgttgggtcctccgccactgtcgacggcgtcgacgtcatcctcttcttccgcatcttcctcgtctgcctgctcttcttcggctgcgttgtcttcgtcgttggcgccatcgaatgcgcacagtgttgcagccacgactcttgcgatagccgcgttgcaacatcaacctctttcgtcgccatcgacagcagctgccgtcgcggccgccacgtcggccgtggctgcggccgcagctacggccaacgcgatggcttctcaattgcaagcagcgcctagtgcccagtcagccgccgctgccgttgctgctgccgccgccgccgccgccgccgccgccgctgctgctgctgccaatctgccggccagcagtaaattgtgcgaaaaaaataagatgttggcttcgttattggccaagacgcccgtgatgccgtcgccgtcgtcgaccaatattgcctcgcccaaaccgtcagcgttgcctcaggagaaattgcctaaggatttgaaggagaaaattcttcagacgccgccagtcagtggaacgtcggctccgggcgcccattgggctggaggctcggtgcaaacccagcccccgacgactatgcaattgcccccgcatccggcgatccaacaacctcagcaacagcaacaacacgttcttaaccagcaacaacagcagcagcaacagcagcagcagcagcagcaacagcaacagcaacagcaacagcaacagcaacaacagcaacgacatccggccatgcaacaatcacagcagcatcagttacaccctcgatctcagcatcttccacaacaacatcagcatttgaacctcggtcagaagcaacagcagcaaccaactcctcaaaccggtggattcttgaattctctcctgaaccggcccatagattccgcctcgggtcccaatattatcggagagtctcaacaacaggccaatcagcagcagcagcagcagcaacaacaacaacaacaacaactatatttagctgctcaacagcctccgcctgtccaacttcagcatcgacccaatcagacggtacagaaattgtcgctcaacaaccaacaacagctttcggcggctatgaactcgtctggtggtttcaacatttctcttcatcctcaacaacaccagcagcagcagcagcagcatcatcaccaccttcaacagcagcagcagcaacaacaacaacaccatcagcagcagcagcagcagcagcagcaacaacaacaacaacaacaacaacaacaacaacagcatcatcaactgcagcatcaactctctggttctatgctggccgatcgtggccttttgcaagctggcggaggaccgggccaacgatccggcatgtcgatccagccgcaacagcagacgtcgcatgccaattccatgattgcagccgccagtttggaaagcagcgatggcagctacagcgttcacgccgactttatgactccgctggacgtccaaatggcttctgtggccggctggggtgacacgccttccatggatccggagctttccgacatcattgagcaggtcatcgacatggatgagcgctacgagagcgattcgatgattttcggcgaattgacatcggtcacgccaccgccagtcgccatccagcccgtcctgtccgttcagtcgtcgcaagcgatcgcttcggtggctcaagcgactgccattgtcggcccactaggcccgcaccttcaaatggacatgtcgaaagagaaactggccatcacggccattcaaaagtcgctcatgtcctacgagaagattcccaccgtagctcaaagtcctccggcctacaatctgcccggctacgcacaacagggtcaaggagcaccgacgagaatgtccactccaacttacggcatgaattcagcaccggccagttcattgcccatggcgaatcaacaactgcaaaccaacttgacgatgccgggagctagaaaacagaaattacccgttcagcaaagacgactggctaatagacaacagcaacagcagcagcagcaacagcagcagcagcaacagcagcagcaacagcaacagcaacagcagcagcagcagtcatcgtcgcaagaacaacaacaacaacaacaacaaccagctcctcagcagcagctactaggcgtcttgctgaatgaatcgtctgtacaacacacccaaggggcacagctctcacccggagccttgcaaattatggatgacctacttaacgcgatcccacccaacatgacgatatccaggtaa

SEQ ID NO: 14 - protein, 2223 aa, Daphnia magna
MLTDTAFLDDAQSLGAIPCESLSSEPCWANMNTLSSGGGGGGGSGGSSNSNSPGLGSNNNNHTTSSASPTTTTTTGNSNSSGGGAGGSNGLTGTSAAAIKKRRKSDTKPLSQINKCLNEKRRREQENVYIEELAELISVSIADVNSLSVKPDKCAILQETVNQIRKIREQEEDGRSSSSSSSSSSSTSSNGSSTNSSGTSSANSGTGGTVGAVGAGGAGGAVGAVGAVGGGGQGNNTTSPGGVTDGGVGPLLQQGDVSSSKPALLDTQLLGTFLLEALDGFLFVVNTEGKTEYVSENVAHFLHYQPQDLVGKSIYNFIHHGDHARFSSSLLPTAIAWPSEMAPTSQNRIGRCFNCRLLIQPLGEQDETMEEKQQRVEHYENMQISAVLQPYPADGGQQQQQPTKKISGAAAAAAAAAAAVGLETSDLELALTSVASGSLAGDPQHCLVCVARRIPSTEKMAAANPTVGGPIVEQFTTKLDPSGKIVAVDVTGVSSPYSSYLSKEALVSCTIQELCYPDDLPVFQAHLQETLHSGCGISSRYRLRLTGASTPMGHRGGAGGGSGGFLVVQTKSKRFIHGDTHETDFIMATHSIIVDDDGEDVDTGNSSSSNTNTNTSRMMLLAAASDTLNDHHRLSESTGSIISQPQQQQQQQQQQQQQQQSNPVLTSVVRHDVISATSFGNSGCSGGATTATTSSTSSSSYSSTFAGLSLGTSGDLLNDFVVPDLFMASPPWDFNNSESSLDDGGSGVALAAASAAASAAVAAAAQITNSHHLQAVTATSSLQLSVPSPLSLIPSGGPLLAGHLPHHSVGGMINWGSPPPSAGAGGVGQRAGSTPCGQMATVMGSSRPSSRQSASSTPRPPSVSSAFSPAPNSVLGVVHPSPVLSPVGATSIHSAAMSCTSGLVTGSTSSSSAGQQQPSPASMTTPFSNNFPFSPLQDPIPQHPATAPQTHNPATPFLDEVRDTKDGIISSGPGGSVSHGHNYLSGGSHHQQQHHHHHQQQQQQQQQQQHATDKQMSALSSLLNCNDAATSSSSSSSSSSSSSSSSSLAESGRLRILLMQRPGNAPPPSAHQQPGHSSSGSSSSSSSTSTSTSTSTSTSTNTNTNTNSSNNNNNNNNNASGNNNSSSVNGSHLLAALGDAEAVKREKDENSGAPSCGSLSVTKGSHGNRILKGLLNQDDGDEADQADDTSNHRFLLTARGNLSGDGVKTSSSAGNNNNNTTNTNNNNTNNNNNMLHKLLNVRSDDDAEQRMGLRKPNELLKKLLKDPEEDHQQASGNGSSSACGGTGSGGTANQLQQFHHQRQQQQQQQQQHQQHQQHQQHQQSQQQQQQNQHHHSDQVSFQEEQLLKSFGFPSPTASSGSSTAATVATGSLANMLATSQMTHLRSPQPPGMSSHCDGLLEFGGVVCSSTTASGMVFGGNAAVGGASGMRGTKRHSEEARDEVKASKEPMLSADHLMMSAGGGGVLHQLLGPPPLSTASTSSSSSASSSSACSSSAALSSSLAPSNAHSVAATTLAIAALQHQPLSSPSTAAAVAAATSAVAAAAATANAMASQLQAAPSAQSAAAAVAAAAAAAAAAAAAAAANLPASSKLCEKNKMLASLLAKTPVMPSPSSTNIASPKPSALPQEKLPKDLKEKILQTPPVSGTSAPGAHWAGGSVQTQPPTTMQLPPHPAIQQPQQQQQHVLNQQQQQQQQQQQQQQQQQQQQQQQQQQQRHPAMQQSQQHQLHPRSQHLPQQHQHLNLGQKQQQQPTPQTGGFLNSLLNRPIDSASGPNIIGESQQQANQQQQQQQQQQQQQLYLAAQQPPPVQLQHRPNQTVQKLSLNNQQQLSAAMNSSGGFNISLHPQQHQQQQQQHHHHLQQQQQQQQQHHQQQQQQQQQQQQQQQQQQQQHHQLQHQLSGSMLADRGLLQAGGGPGQRSGMSIQPQQQTSHANSMIAAASLESSDGSYSVHADFMTPLDVQMASVAGWGDTPSMDPELSDIIEQVIDMDERYESDSMIFGELTSVTPPPVAIQPVLSVQSSQAIASVAQATAIVGPLGPHLQMDMSKEKLAITAIQKSLMSYEKIPTVAQSPPAYNLPGYAQQGQGAPTRMSTPTYGMNSAPASSLPMANQQLQTNLTMPGARKQKLPVQQRRLANRQQQQQQQQQQQQQQQQQQQQQQQQQQSSSQEQQQQQQQPAPQQQLLGVLLNESSVQHTQGAQLSPGALQIMDDLLNAIPPNMTISR

SEQ ID NO: 15 - DNA, 101 bp, Artificial
  Synthetic DNA
ctagtccattttccattcccatgtgcagaatgtgcgaaaaacgttgcacgtcctctcgatggcgtcgaaaatcgttgcacggccgccacgcgaactctgct

SEQ ID NO: 16 - DNA, 101 bp, Artificial
  Synthetic DNA
ctagagcagagttcgcgtggcggccgtgcaacgattttcgacgccatcgagaggacgtgcaacgtttttcgcacattctgcacatgggaatggaaaatgga

SEQ ID NO: 17 - DNA, 78 bp, Artificial
  Synthetic DNA
aataggggttccgcgcacatttccccgaaaagtgccacctattaccctgttatccctaggtccttttcatcacgtgct

SEQ ID NO: 18 - DNA, 78 bp, Artificial
  Synthetic DNA
tatttttataggttaatgtcatgataataatggtttcttatagggataacagggtaataggacggatcgcttgcctgt

SEQ ID NO: 19 - DNA, 72 bp, Artificial
  Synthetic DNA
tttgcgtccatccaaaaaaaaagtaagaatttttgaaaggggatccaacaaaatggacaaaatgagcgagac

SEQ ID NO: 20 - DNA, 60 bp, Artificial
  Synthetic DNA
cggttagagcggatgtgggaggagggcgtgaatgtaagcttctatgcactgttggttcca

SEQ ID NO: 21 - DNA, 40 bp, Artificial
  Synthetic DNA
cccccccgggaacaaaatggcagcaccagagacgggcaac

SEQ ID NO: 22 - DNA, 35 bp, Artificial
  Synthetic DNA
ccccgaattcctcatcgcagcgtgctggtcagggt

SEQ ID NO: 23 - DNA, 73 bp, Artificial
  Synthetic DNA
tttgaaaattcgaattcaaccctcactaaagggcggccgcactagtaaaaacatgctgacggataccgcattc

SEQ ID NO: 24 - DNA, 69 bp, Artificial
  Synthetic DNA
cttgattggagacttgaccaaacctctggcgaagaattgttaattaattacctggatatcgtcatgttg

SEQ ID NO: 25 - DNA, 43 bp, Artificial
  Synthetic DNA
caaagaaaatacgcagggcccgcggcacgtgtgtgcatcccat

SEQ ID NO: 26 - DNA, 49 bp, Artificial
  Synthetic DNA
ctagtcaaagaaaatacgcagggcccgcggcacgtgtgtgcatcccatt

SEQ ID NO: 27 - DNA, 49 bp, Artificial
  Synthetic DNA
ctagaatgggatgcacacacgtgccgcgggccctgcgtattttctttga

SEQ ID NO: 28 - DNA, 43 bp, Artificial
  Synthetic DNA
caaagaaaatacgcacacgcggcggaggccttgtgcatcccat

SEQ ID NO: 29 - DNA, 49 bp, Artificial
  Synthetic DNA
ctagtcaaagaaaatacgcacacgcggcggaggccttgtgcatcccatt

SEQ ID NO: 30 - DNA, 49 bp, Artificial
  Synthetic DNA
ctagaatgggatgcacaaggcctccgccgcgtgtgcgtattttctttga

SEQ ID NO: 31 - DNA, 43 bp, Artificial
  Synthetic DNA
caaagaaaatacgcagggcccgcggaggccttgtgcatcccat

SEQ ID NO: 32 - DNA, 49 bp, Artificial
  Synthetic DNA
ctagtcaaagaaaatacgcagggcccgcggaggccttgtgcatcccatt

SEQ ID NO: 33 - DNA, 49 bp, Artificial
  Synthetic DNA
ctagaatgggatgcacaaggcctccgcgggccctgcgtattttctttga

SEQ ID NO: 34 - DNA, 22 bp, Daphnia magna
gcacacgcggcggcacgtgtgt

SEQ ID NO: 35 - DNA, 28 bp, Artificial
  Synthetic DNA
ctagtgcacacgcggcggcacgtgtgtt

SEQ ID NO: 36 - DNA, 28 bp, Artificial
  Synthetic DNA
ctagaacacacgtgccgccgcgtgtgca

SEQ ID NO: 37 - DNA, 36 bp, Daphnia magna
aaaatacgcacacgcggcggcacgtgtgtgcatccc

SEQ ID NO: 38 - DNA, 42 bp, Artificial
  Synthetic DNA
ctagtaaaatacgcacacgcggcggcacgtgtgtgcatccct

SEQ ID NO: 39 - DNA, 42 bp, Artificial
  Synthetic DNA
ctagagggatgcacacacgtgccgccgcgtgtgcgtatttta

SEQ ID NO: 40 - DNA, 43 bp, Artificial
  Synthetic DNA
caaagaaaatactaccacgcggcggcacgtgtgtgcatcccat

SEQ ID NO: 41 - DNA, 49 bp, Artificial
  Synthetic DNA
ctagtcaaagaaaatactaccacgcggcggcacgtgtgtgcatcccatt

SEQ ID NO: 42 - DNA, 49 bp, Artificial
  Synthetic DNA
ctagaatgggatgcacacacgtgccgccgcgtggtagtattttctttga

SEQ ID NO: 43 - DNA, 43 bp, Artificial
  Synthetic DNA
caaagaaaatacgcacacgcggcggcacgtggtggcatcccat

SEQ ID NO: 44 - DNA, 49 bp, Artificial
  Synthetic DNA
ctagtcaaagaaaatacgcacacgcggcggcacgtggtggcatcccatt

SEQ ID NO: 45 - DNA, 49 bp, Artificial
  Synthetic DNA
ctagaatgggatgccaccacgtgccgccgcgtgtgcgtattttctttga

SEQ ID NO: 46 - DNA, 43 bp, Artificial
  Synthetic DNA
caaagaaaatactaccacgcggcggcacgtggtggcatcccat

SEQ ID NO: 47 - DNA, 49 bp, Artificial
  Synthetic DNA
ctagtcaaagaaaatactaccacgcggcggcacgtggtggcatcccatt

SEQ ID NO: 48 - DNA, 49 bp, Artificial
  Synthetic DNA
ctagaatgggatgccaccacgtgccgccgcgtggtagtattttctttga

SEQ ID NO: 49 - DNA, 43 bp, Artificial
  Synthetic DNA
caaagaaaatacgcacacgcgtattcacgtgtgtgcatcccat

SEQ ID NO: 50 - DNA, 49 bp, Artificial
  Synthetic DNA
ctagtcaaagaaaatacgcacacgcgtattcacgtgtgtgcatcccatt

SEQ ID NO: 51 - DNA, 49 bp, Artificial
  Synthetic DNA
ctagaatgggatgcacacacgtgaatacgcgtgtgcgtattttctttga

SEQ ID NO: 52 - DNA, 43 bp, Artificial
  Synthetic DNA
caaagaaaatactaccacgcgtattcacgtggtggcatcccat

SEQ ID NO: 53 - DNA, 49 bp, Artificial
  Synthetic DNA
ctagtcaaagaaaatactaccacgcgtattcacgtggtggcatcccatt

SEQ ID NO: 54 - DNA, 49 bp, Artificial
  Synthetic DNA
ctagaatgggatgccaccacgtgaatacgcgtggtagtattttctttga